European Patent Application EP 4 400 588 A1, published July 17, 2024. Title: RECOMBINANT MICROORGANISM USED FOR PRODUCING CDP-CHOLINE, AND METHOD FOR PRODUCING CDP-CHOLINE USING SAID RECOMBINANT MICROORGANISM. Applicant: 協和発酵バイオ株式会社. Application EP 22 867 449.5, filed September 9, 2022. The sequence listing filed with the application follows.

SEQUENCE LISTING (14 sequences)

SEQ ID NO: 1 - DNA, 690 bp, Streptococcus pneumoniae
  source 1..690: mol_type = genomic DNA
gtgaaagccattatcttagcagcgggattgggaactcgcttgcgtcctatgactgaaaatacccctaaagccttggttcaggttaatcaaaaacctttgattgaataccaaattgagtttctcaaagaaaaaggaatcaatgacatcatcatcattgttggttatcttaaagaacaattcgattacttaaaagaaaaatacggtgttcgcctcgttttcaatgataaatacgctgactacaataacttttactctctctatcttgtaaaagaagaattggccaacagctatgttattgatgctgacaattatctctttaaaaatatgttccgcaatgatttgacacgttcgacttattttagtgtttatcgtgaagattgtaccaacgaatggttcttggtctatggagatgactacaaggttcaagacattattgttgatagcaaggcaggtcgcatccttagtggtgtatccttctgggatgctccaactgcagaaaagattgtcagctttatcgacaaggcttatgcaagtggtgaatttgttgatctctattgggacaatatggttaaggataatatcaaagagctagatgtctatgttgaagaattagaaggcaatagcatttatgagatcgatagtgtccaagactatcgtaaattagaagaaattcttaaaaacgaaaattaa

SEQ ID NO: 2 - DNA, 34 bp, synthetic construct
  source 1..34: mol_type = other DNA
  misc_feature 1..34: note = Description of the artificial sequence: base sequence ofprimer_Fw for cloning SplicC
ggagatatacatatgaaagccattatcttagcag

SEQ ID NO: 3 - DNA, 42 bp, synthetic construct
  source 1..42: mol_type = other DNA
  misc_feature 1..42: note = Description of the artificial sequence: base sequence ofprimer_Rv for cloning SplicC
gtggtggtgctcgagattttcgtttttaagaatttcttctaa

SEQ ID NO: 4 - DNA, 19 bp, synthetic construct
  source 1..19: mol_type = other DNA
  misc_feature 1..19: note = Description of the artificial sequence: base sequence ofprimer_Fw for Inverse pET21a
ctcgagcaccaccaccacc

SEQ ID NO: 5 - DNA, 30 bp, synthetic construct
  source 1..30: mol_type = other DNA
  misc_feature 1..30: note = Description of the artificial sequence: base sequence ofprimer_Rv for Inverse pET21a
catatgtatatctccttcttaaagttaaac

SEQ ID NO: 6 - protein, 237 aa, synthetic construct
  REGION 1..237: note = Description of the artificial sequence: amino acid sequence ofthe insert of pET21a-SplicC
VKAIILAAGLGTRLRPMTENTPKALVQVNQKPLIEYQIEFLKEKGINDIIIIVGYLKEQFDYLKEKYGVRLVFNDKYADYNNFYSLYLVKGELANSYVIDADNYLFKNMFRNDLTRSTYFSVYREDCTNEWFLVYGDDYKVQDIIVDSKAGRILSGVSFWDAPTAEKIVSFIDKAYASGEFVDLYWDNMVKDNIKELDVYVEELEGNSIYEIDSVQDYRKLEEILKNENLEHHHHHH

SEQ ID NO: 7 - DNA, 702 bp, Lactobacillus salivarius
  source 1..702: mol_type = genomic DNA
atgagtaaagttaaaagagcaattataatggctgctggctatggtacaaggttaagaccaataactttatctacgcctaaaccattgataaaagtaaatggaatcagaatgattgaatcagttatagaggcattgctaaaaaatgatataagagaaatatatgttgtgacaggttatttggttgaaaaatttgactttttaggagaaaagtatccagaagtaacccttatatataatccatattatagtaaatataataatatttcttcattatacgtagctagagaccatttgaaagatgtaattattttagatggagatcaaatcattaaaaatgataaaatcttagatcctaattttgaaaaatctgggtataactgtgtatggagtgaaggatacacggatgaatggcttttacaagtagaaaaaaatacaatagttagttgtagcagaaatggtggagaaaaaggttggcgcttgtatagcatttctcgttggaatcaagaagatggtcaaaaattgaaagcagacttggaatatcaatttgaagtagaaaaaaattatgatatttattgggatgatgtggcattattttgctcccctcaaaattatgatttaggtattagagaaatgaacttagatgatgttatagagatagatacgattgatgaattaagattagttgataaaagctacgactag

SEQ ID NO: 8 - DNA, 32 bp, synthetic construct
  source 1..32: mol_type = other DNA
  misc_feature 1..32: note = Description of the artificial sequence: base sequence ofprimer_Fw for cloning LslicC
ggagatatacatatgagtaaagttaaaagagc

SEQ ID NO: 9 - DNA, 36 bp, synthetic construct
  source 1..36: mol_type = other DNA
  misc_feature 1..36: note = Description of the artificial sequence: base sequence ofprimer_Rv for cloning LslicC
gtggtggtgctcgaggtcgtcgtagcttttatcaac

SEQ ID NO: 10 - protein, 242 aa, synthetic construct
  REGION 1..242: note = Description of the artificial sequence: amino acid sequence ofthe insert of pET21a-LslicC
MSKVKRAIIMAAGYGTRLRPITLSTPKPLIKVNGIRMIESVIEALLKNDIREIYVVTGYLAEKFDFLGEKYPEVTLIYNPYYSKYNNISSLYVARDHLKDVIILDGDQIIKNDKILDPNFEKSGYNCVWSEGYTDEWLLQVEKNTIVSCSRNGGEKGWRLYSISRWNQEDGQKLKADLEYQFEVEKNYDIYWDDVALFCSPQNYDLGVREMNLDDVIEIDTIDELRLVDKSYDDLEHHHHHH

SEQ ID NO: 11 - DNA, 714 bp, Anaerococcus hydrogenalis
  source 1..714: mol_type = genomic DNA
atgtataaggtaaaaagggcaataattatggcagcaggctttggaaataggatgaaacctgtgaccttagatacgcccaaacccttaataaaagttaatggtaagagaatgattgatactataattgatggtttgcataaaaatggtatagatgaaatttatcttgtggttggatatttatcagaaaaattccaggaattattggaaaaatatccaaatttaaattttataaaaaatccctattatgatacttgtaacaacatttcttctttatatgtagctagaaatttgatttcaaatgcaataattttggatggggaccaaattatttataatgatgaaattttaagtccaaattttgaaaagtctggttacaatagtgtatggacaagttcttatactgacgagtggctacaaaatgtagaagatgggaaagttatttcttgtagtaaaaccggtggtaaaaacggttggcaattatatagcgtttctcgttggaatgaaaaagacgggaaaaaattgaaacattttatagaattagaatttgaaaataataacaggcaaatttattgggacgatgtggccctattttgccatccggatgaatttgatttgggaattttcccaatgaaaaaagaagatattgttgaaattgataatttttctgaacttttggccatagacccaagttataaaaattatccccaaaaatag

SEQ ID NO: 12 - DNA, 32 bp, synthetic construct
  source 1..32: mol_type = other DNA
  misc_feature 1..32: note = Description of the artificial sequence: base sequence ofprimer_Fw for cloning AhlicC
ggagatatacatatgtataaggtaaaaagggc

SEQ ID NO: 13 - DNA, 42 bp, synthetic construct
  source 1..42: mol_type = other DNA
  misc_feature 1..42: note = Description of the artificial sequence: base sequence ofprimer_Rv for cloning AhlicC
gtggtggtgctcgagtttttggggataatttttataacttgg

SEQ ID NO: 14 - protein, 245 aa, synthetic construct
  REGION 1..245: note = Description of the artificial sequence: amino acid sequence ofthe insert of pET21a-AhlicC
MYKVKRAIIMAAGFGNRMKPVTLDTPKPLIKVNGKRMIDTIIDGLHKNGIDEIYLVVGYLSEKFQELLEKYPNLNFIKNPYYDTCNNISSLYVARNLISNAIILDGDQIIYNDEILSPNFEKSGYNSVWTSSYTDEWLQNVEDGKVISCSKTGGKNGWQLYSVSRWNEKDGKKLKHFIELEFENNNRQIYWDDVALFCHPDEFDLGIFPMKKEDIVEIDNFSELLAIDPSYKNYPQKLEHHHHHH